European Patent Specification EP 3 664 603 B1, published January 3, 2024. Title: IMMUNODEFICIENT MICE TRANSGENICALLY EXPRESSING HUMAN INTERLEUKIN 15. Applicant: The Jackson Laboratory. The sequence listing filed with the application follows.

SEQUENCE LISTING (2 sequences)

SEQ ID NO: 1 - protein, 162 aa, Homo sapiens
MRISKPHLRSISIQCYLCLLLNSHFLTEAGIHVFILGCFSAGLPKTEANWVNVISDLKKIEDLIQSMHIDATLYTESDVHPSCKVTAMKCFLLELQVISLESGDASIHDTVENLIILANNSLSSNGNVTESGCKECEELEEKNIKEFLQSFVHIVQMFINTS

SEQ ID NO: 2 - DNA, 486 bp, Homo sapiens
atgagaatttcgaaaccacatttgagaagtatttccatccagtgctacttgtgtttacttctaaacagtcattttctaactgaagctggcattcatgtcttcattttgggctgtttcagtgcagggcttcctaaaacagaagccaactgggtgaatgtaataagtgatttgaaaaaaattgaagatcttattcaatctatgcatattgatgctactttatatacggaaagtgatgttcaccccagttgcaaagtaacagcaatgaagtgctttctcttggagttacaagttatttcacttgagtccggagatgcaagtattcatgatacagtagaaaatctgatcatcctagcaaacaacagtttgtcttctaatgggaatgtaacagaatctggatgcaaagaatgtgaggaactggaggaaaaaaatattaaagaatttttgcagagttttgtacatattgtccaaatgttcatcaacacttct